European Patent Application EP 4 703 474 A1, published March 4, 2026. Title: ANTI-LRRC15 ANTIBODY. Applicant: DAIICHI SANKYO COMPANY, LIMITED. Application EP 24747371.3, filed January 26, 2024. The sequence listing filed with the application follows.

SEQUENCE LISTING (73 sequences)

SEQ ID NO: 1 - protein, 581 aa, Homo sapiens
MPLKHYLLLLVGCQAWGAGLAYHGCPSECTCSRASQVECTGARIVAVPTPLPWNAMSLQILNTHITELNESPFLNISALIALRIEKNELSRITPGAFRNLGSLRYLSLANNKLQVLPIGLFQGLDSLESLLLSSNQLLQIQPAHFSQCSNLKELQLHGNHLEYIPDGAFDHLVGLTKLNLGKNSLTHISPRVFQHLGNLQVLRLYENRLTDIPMGTFDGLVNLQELALQQNQIGLLSPGLFHNNHNLQRLYLSNNHISQLPPSVFMQLPQLNRLTLFGNSLKELSPGIFGPMPNLRELWLYDNHISSLPDNVFSNLRQLQVLILSRNQISFISPGAFNGLTELRELSLHTNALQDLDGNVFRMLANLQNISLQNNRLRQLPGNIFANVNGLMAIQLQNNQLENLPLGIFDHLGKLCELRLYDNPWRCDSDILPLRNWLLLNQPRLGTDTVPVCFSPANVRGQSLIIINVNVAVPSVHVPEVPSYPETPWYPDTPSYPDTTSVSSTTELTSPVEDYTDLTTIQVTDDRSVWGMTQAQSGLAIAAIVIGIVALACSLAACVGCCCCKKRSQAVLMQMKAPNEC

SEQ ID NO: 2 - protein, 517 aa, Homo sapiens
YHGCPSECTCSRASQVECTGARIVAVPTPLPWNAMSLQILNTHITELNESPFLNISALIALRIEKNELSRITPGAFRNLGSLRYLSLANNKLQVLPIGLFQGLDSLESLLLSSNQLLQIQPAHFSQCSNLKELQLHGNHLEYIPDGAFDHLVGLTKLNLGKNSLTHISPRVFQHLGNLQVLRLYENRLTDIPMGTFDGLVNLQELALQQNQIGLLSPGLFHNNHNLQRLYLSNNHISQLPPSVFMQLPQLNRLTLFGNSLKELSPGIFGPMPNLRELWLYDNHISSLPDNVFSNLRQLQVLILSRNQISFISPGAFNGLTELRELSLHTNALQDLDGNVFRMLANLQNISLQNNRLRQLPGNIFANVNGLMAIQLQNNQLENLPLGIFDHLGKLCELRLYDNPWRCDSDILPLRNWLLLNQPRLGTDTVPVCFSPANVRGQSLIIINVNVAVPSVHVPEVPSYPETPWYPDTPSYPDTTSVSSTTELTSPVEDYTDLTTIQVTDDRSVWGMTQAQSG

SEQ ID NO: 3 - protein, 544 aa, Homo sapiens
MPLKHYLLLLVGCQAWGAGLAYHGCPSECTCSRASQVECTGARIVAVPTPLPWNAMSLQILNTHITELNESPFLNISALIALRIEKNELSRITPGAFRNLGSLRYLSLANNKLQVLPIGLFQGLDSLESLLLSSNQLLQIQPAHFSQCSNLKELQLHGNHLEYIPDGAFDHLVGLTKLNLGKNSLTHISPRVFQHLGNLQVLRLYENRLTDIPMGTFDGLVNLQELALQQNQIGLLSPGLFHNNHNLQRLYLSNNHISQLPPSVFMQLPQLNRLTLFGNSLKELSPGIFGPMPNLRELWLYDNHISSLPDNVFSNLRQLQVLILSRNQISFISPGAFNGLTELRELSLHTNALQDLDGNVFRMLANLQNISLQNNRLRQLPGNIFANVNGLMAIQLQNNQLENLPLGIFDHLGKLCELRLYDNPWRCDSDILPLRNWLLLNQPRLGTDTVPVCFSPANVRGQSLIIINVNVAVPSVHVPEVPSYPETPWYPDTPSYPDTTSVSSTTELTSPVEDYTDLTTIQVTDDRSVWGMTQAQSGHHHHHH

SEQ ID NO: 4 - protein, 581 aa, Macaca fascicularis
MPLKHYLLLLVGCQAWGAGLAYYGCPSECTCSRASQVECTGARIVAVPTPLPWNAMSLQILNTHITELSESPFLNISALIALRIEKNELSHIMPGAFRNLGSLRYLSLANNKLQVLPIGLFQGLDSLESLLLSSNQLVQIQPAHFSQCSNLKELQLHGNHLEYIPDGAFDHLVGLTKLNLGKNSLTHISPRVFQHLGNLQVLRLYENRLTDIPMGTFDGLVNLQELALQQNQIGLLSPGLFHNNHNLQRLYLSNNHISQLPPSIFMQLPQLNRLTLFGNSLKELSPGIFGPMPNLRELWLYDNHITSLPDNVFSNLRQLQVLILSRNQISFISPGAFNGLTELRELSLHTNALQDLDGNVFRMLANLQNISLQNNRLRQLPGNIFANVNGLMTIQLQNNQLENLPLGIFDHLGKLCELRLYDNPWRCDSDILPLRNWLLLNQPRLGTDTVPVCFSPANVRGQSLIIINVNVAVPSVHVPEVPSYPETSWYPDTSSYPDTTSISSTTELTSPVEDYTDLTTIQVTDDRSVWGMTQAQSGLAIAAIVIGIVALACSLAACIGCCCCKKRSQAVLMQMKAPNEC

SEQ ID NO: 5 - protein, 517 aa, Macaca fascicularis
YYGCPSECTCSRASQVECTGARIVAVPTPLPWNAMSLQILNTHITELSESPFLNISALIALRIEKNELSHIMPGAFRNLGSLRYLSLANNKLQVLPIGLFQGLDSLESLLLSSNQLVQIQPAHFSQCSNLKELQLHGNHLEYIPDGAFDHLVGLTKLNLGKNSLTHISPRVFQHLGNLQVLRLYENRLTDIPMGTFDGLVNLQELALQQNQIGLLSPGLFHNNHNLQRLYLSNNHISQLPPSIFMQLPQLNRLTLFGNSLKELSPGIFGPMPNLRELWLYDNHITSLPDNVFSNLRQLQVLILSRNQISFISPGAFNGLTELRELSLHTNALQDLDGNVFRMLANLQNISLQNNRLRQLPGNIFANVNGLMTIQLQNNQLENLPLGIFDHLGKLCELRLYDNPWRCDSDILPLRNWLLLNQPRLGTDTVPVCFSPANVRGQSLIIINVNVAVPSVHVPEVPSYPETSWYPDTSSYPDTTSISSTTELTSPVEDYTDLTTIQVTDDRSVWGMTQAQSG

SEQ ID NO: 6 - protein, 544 aa, Macaca fascicularis
MPLKHYLLLLVGCQAWGAGLAYYGCPSECTCSRASQVECTGARIVAVPTPLPWNAMSLQILNTHITELSESPFLNISALIALRIEKNELSHIMPGAFRNLGSLRYLSLANNKLQVLPIGLFQGLDSLESLLLSSNQLVQIQPAHFSQCSNLKELQLHGNHLEYIPDGAFDHLVGLTKLNLGKNSLTHISPRVFQHLGNLQVLRLYENRLTDIPMGTFDGLVNLQELALQQNQIGLLSPGLFHNNHNLQRLYLSNNHISQLPPSIFMQLPQLNRLTLFGNSLKELSPGIFGPMPNLRELWLYDNHITSLPDNVFSNLRQLQVLILSRNQISFISPGAFNGLTELRELSLHTNALQDLDGNVFRMLANLQNISLQNNRLRQLPGNIFANVNGLMTIQLQNNQLENLPLGIFDHLGKLCELRLYDNPWRCDSDILPLRNWLLLNQPRLGTDTVPVCFSPANVRGQSLIIINVNVAVPSVHVPEVPSYPETSWYPDTSSYPDTTSISSTTELTSPVEDYTDLTTIQVTDDRSVWGMTQAQSGHHHHHH

SEQ ID NO: 7 - protein, 579 aa, Mus musculus
MPLKHYLLLLVSCQAWAAGLAYYGCPSECTCSRASQVECTGAQIVAMPSPLPWNAMSLQILNTHITELPEDKFLNISALIALKMEKNELANIMPGAFRNLGSLRHLSLANNKLKNLPVRLFQDVNNLETLLLSNNQLVQIQPAQFSQFSNLKELQLYGNNLEYIPEGVFDHLVGLTKLNLGNNGFTHLSPRVFQHLGNLQVLRLYENRLSDIPMGTFDALGNLQELALQENQIGTLSPGLFHNNRNLQRLYLSNNHISHLPPGIFMQLPHLNKLTLFGNSLKELSPGVFGPMPNLRELWLYNNHITSLPDNAFSHLNQLQVLILSHNQLSYISPGAFNGLTNLRELSLHTNALQDLDGNVFRSLANLRNVSLQNNRLRQLPGSIFANVNGLMTIQLQNNNLENLPLGIFDHLGNLCELRLYDNPWRCDSNILPLHDWLILNRARLGTDTLPVCSSPASVRGQSLVIINVNFPGPSVQGPETPEVSSYPDTSSYPDSTSISSTTEITRSTDDDYTDLNTIEPIDDRNTWGMTDAQSGLAIAAIVIGIIALACSLAACICCCCCKKRSQAVLMQMKAPNEC

SEQ ID NO: 8 - protein, 515 aa, Mus musculus
YYGCPSECTCSRASQVECTGAQIVAMPSPLPWNAMSLQILNTHITELPEDKFLNISALIALKMEKNELANIMPGAFRNLGSLRHLSLANNKLKNLPVRLFQDVNNLETLLLSNNQLVQIQPAQFSQFSNLKELQLYGNNLEYIPEGVFDHLVGLTKLNLGNNGFTHLSPRVFQHLGNLQVLRLYENRLSDIPMGTFDALGNLQELALQENQIGTLSPGLFHNNRNLQRLYLSNNHISHLPPGIFMQLPHLNKLTLFGNSLKELSPGVFGPMPNLRELWLYNNHITSLPDNAFSHLNQLQVLILSHNQLSYISPGAFNGLTNLRELSLHTNALQDLDGNVFRSLANLRNVSLQNNRLRQLPGSIFANVNGLMTIQLQNNNLENLPLGIFDHLGNLCELRLYDNPWRCDSNILPLHDWLILNRARLGTDTLPVCSSPASVRGQSLVIINVNFPGPSVQGPETPEVSSYPDTSSYPDSTSISSTTEITRSTDDDYTDLNTIEPIDDRNTWGMTDAQSG

SEQ ID NO: 9 - protein, 542 aa, Mus musculus
MPLKHYLLLLVSCQAWAAGLAYYGCPSECTCSRASQVECTGAQIVAMPSPLPWNAMSLQILNTHITELPEDKFLNISALIALKMEKNELANIMPGAFRNLGSLRHLSLANNKLKNLPVRLFQDVNNLETLLLSNNQLVQIQPAQFSQFSNLKELQLYGNNLEYIPEGVFDHLVGLTKLNLGNNGFTHLSPRVFQHLGNLQVLRLYENRLSDIPMGTFDALGNLQELALQENQIGTLSPGLFHNNRNLQRLYLSNNHISHLPPGIFMQLPHLNKLTLFGNSLKELSPGVFGPMPNLRELWLYNNHITSLPDNAFSHLNQLQVLILSHNQLSYISPGAFNGLTNLRELSLHTNALQDLDGNVFRSLANLRNVSLQNNRLRQLPGSIFANVNGLMTIQLQNNNLENLPLGIFDHLGNLCELRLYDNPWRCDSNILPLHDWLILNRARLGTDTLPVCSSPASVRGQSLVIINVNFPGPSVQGPETPEVSSYPDTSSYPDSTSISSTTEITRSTDDDYTDLNTIEPIDDRNTWGMTDAQSGHHHHHH

SEQ ID NO: 10 - protein, 578 aa, Rattus norvegicus
MPLKHYLLLLVGCQAWALGLAYYGCPSECTCSRASQVECTGARIVAMPTPLPWNAMSLQVVNTHITELPENLFLNISALIALKMEKNELSTIMPGAFRNLGSLRYLSLANNKLRMLPIRVFQDVNNLESLLLSNNQLVQIQPAQFSQFSNLRELQLHGNNLESIPEEAFDHLVGLTKLNLGRNSFTHLSPRLFQHLGNLQVLRLHENRLSDIPMGTFDALGNLQELALQENQIGTLSPGLFHNNRNLQRLYLSNNHISQLPPGIFMQLPQLNKLTLFGNSLRELSPGVFGPMPNLRELWLYNNHITSLADNTFSHLNQLQVLILSHNQLTYISPGAFNGLTNLRELSLHTNALQDLDSNVFRSLANLQNISLQSNRLRQLPGSIFANVNGLTTIQLQNNNLENLPLGIFDHLVNLCELRLYDNPWRCDSDILPLHNWLLLNRARLGTDTLPVCSSPANVRGQSLVIININFPGPSVQGPETPEVPSYPDTPSYPDTTSVSSTTEITSAVDDYTDLTTIEATDDRNTWGMTEAQSGLAIAAIVIGIIALACSLAACICCCCCKKRSQAVLMQMKAPNEC

SEQ ID NO: 11 - protein, 514 aa, Rattus norvegicus
YYGCPSECTCSRASQVECTGARIVAMPTPLPWNAMSLQVVNTHITELPENLFLNISALIALKMEKNELSTIMPGAFRNLGSLRYLSLANNKLRMLPIRVFQDVNNLESLLLSNNQLVQIQPAQFSQFSNLRELQLHGNNLESIPEEAFDHLVGLTKLNLGRNSFTHLSPRLFQHLGNLQVLRLHENRLSDIPMGTFDALGNLQELALQENQIGTLSPGLFHNNRNLQRLYLSNNHISQLPPGIFMQLPQLNKLTLFGNSLRELSPGVFGPMPNLRELWLYNNHITSLADNTFSHLNQLQVLILSHNQLTYISPGAFNGLTNLRELSLHTNALQDLDSNVFRSLANLQNISLQSNRLRQLPGSIFANVNGLTTIQLQNNNLENLPLGIFDHLVNLCELRLYDNPWRCDSDILPLHNWLLLNRARLGTDTLPVCSSPANVRGQSLVIININFPGPSVQGPETPEVPSYPDTPSYPDTTSVSSTTEITSAVDDYTDLTTIEATDDRNTWGMTEAQSG

SEQ ID NO: 12 - protein, 541 aa, Rattus norvegicus
MPLKHYLLLLVGCQAWALGLAYYGCPSECTCSRASQVECTGARIVAMPTPLPWNAMSLQVVNTHITELPENLFLNISALIALKMEKNELSTIMPGAFRNLGSLRYLSLANNKLRMLPIRVFQDVNNLESLLLSNNQLVQIQPAQFSQFSNLRELQLHGNNLESIPEEAFDHLVGLTKLNLGRNSFTHLSPRLFQHLGNLQVLRLHENRLSDIPMGTFDALGNLQELALQENQIGTLSPGLFHNNRNLQRLYLSNNHISQLPPGIFMQLPQLNKLTLFGNSLRELSPGVFGPMPNLRELWLYNNHITSLADNTFSHLNQLQVLILSHNQLTYISPGAFNGLTNLRELSLHTNALQDLDSNVFRSLANLQNISLQSNRLRQLPGSIFANVNGLTTIQLQNNNLENLPLGIFDHLVNLCELRLYDNPWRCDSDILPLHNWLLLNRARLGTDTLPVCSSPANVRGQSLVIININFPGPSVQGPETPEVPSYPDTPSYPDTTSVSSTTEITSAVDDYTDLTTIEATDDRNTWGMTEAQSGHHHHHH

SEQ ID NO: 13 - protein, 587 aa, Homo sapiens
MPLDKAMPLKHYLLLLVGCQAWGAGLAYHGCPSECTCSRASQVECTGARIVAVPTPLPWNAMSLQILNTHITELNESPFLNISALIALRIEKNELSRITPGAFRNLGSLRYLSLANNKLQVLPIGLFQGLDSLESLLLSSNQLLQIQPAHFSQCSNLKELQLHGNHLEYIPDGAFDHLVGLTKLNLGKNSLTHISPRVFQHLGNLQVLRLYENRLTDIPMGTFDGLVNLQELALQQNQIGLLSPGLFHNNHNLQRLYLSNNHISQLPPSVFMQLPQLNRLTLFGNSLKELSPGIFGPMPNLRELWLYDNHISSLPDNVFSNLRQLQVLILSRNQISFISPGAFNGLTELRELSLHTNALQDLDGNVFRMLANLQNISLQNNRLRQLPGNIFANVNGLMAIQLQNNQLENLPLGIFDHLGKLCELRLYDNPWRCDSDILPLRNWLLLNQPRLGTDTVPVCFSPANVRGQSLIIINVNVAVPSVHVPEVPSYPETPWYPDTPSYPDTTSVSSTTELTSPVEDYTDLTTIQVTDDRSVWGMTQAQSGLAIAAIVIGIVALACSLAACVGCCCCKKRSQAVLMQMKAPNEC

SEQ ID NO: 14 - DNA, 369 bp, Rattus norvegicus
  source 1..369: mol_type = unassigned DNA
gaggtgcagctggtggagtctaatggagccttagtgcagcctggaaggtccctaaaactctcctgtgcagcctcagggttcaccttccgtgactattacatggcctgggtccgccaggctccatcgaaggggctggagtgggtcgcatccattggttttgatgaaagtcgcacttactatcgagactccgtgaagggccgattcactatctccagagatgatgtaaaaagcaccctatacctacaactggacagtctgaggtctgaggacacggccacttattactgtacaagacatggggtttcttactacagtggtgacaattggtttgcctactggggccaaggcgctctggtcattgtctcttca

SEQ ID NO: 15 - protein, 123 aa, Rattus norvegicus
EVQLVESNGALVQPGRSLKLSCAASGFTFRDYYMAWVRQAPSKGLEWVASIGFDESRTYYRDSVKGRFTISRDDVKSTLYLQLDSLRSEDTATYYCTRHGVSYYSGDNWFAYWGQGALVIVSS

SEQ ID NO: 16 - DNA, 342 bp, Rattus norvegicus
  source 1..342: mol_type = unassigned DNA
gacattgtgatgacccaatctccatcctctctggctgtgtcagcaggagagacggtcattataaactgcaagtccagtcagggtcttttatacagtggagaccaaaagaactacttggcctggtaccagcagaaaccagggcagtctcctaaactgctgatctactgggcatctactaggcaatctggtgtccctgatcgcttcataggcagtggatctgggacagacttcactctgaccatcagcagtgtgcagggagaagatctggcaatttattactgtcagcagtattatgatcctccgtacacgtttggagctgggaccaagctggaactgaaacgg

SEQ ID NO: 17 - protein, 114 aa, Rattus norvegicus
DIVMTQSPSSLAVSAGETVIINCKSSQGLLYSGDQKNYLAWYQQKPGQSPKLLIYWASTRQSGVPDRFIGSGSGTDFTLTISSVQGEDLAIYYCQQYYDPPYTFGAGTKLELKR

SEQ ID NO: 18 - DNA, 449 bp, Homo sapiens
  source 1..449: mol_type = genomic DNA
gcctccggactctagagccaccatggtgctgcagacccaggtgttcatctccctgctgctgtggatctccggcgcgtacggcgatatcgtgatgattaaacgtacggtggccgccccctccgtgttcatcttccccccctccgacgagcagctgaagtccggcaccgcctccgtggtgtgcctgctgaataacttctaccccagagaggccaaggtgcagtggaaggtggacaacgccctgcagtccgggaactcccaggagagcgtgaccgagcaggacagcaaggacagcacctacagcctgagcagcaccctgaccctgagcaaagccgactacgagaagcacaaggtgtacgcctgcgaggtgacccaccagggcctgagctcccccgtcaccaagagcttcaacaggggggagtgttaggggcccgtttaaacgggggaggcta

SEQ ID NO: 19 - DNA, 1117 bp, Homo sapiens
  source 1..1117: mol_type = genomic DNA
gggtctagagccaccatgaaacacctgtggttcttcctcctgctggtggcagctcccagatgggtgctgagccaggtgcaattgtgcaggcggttagctcagcctccaccaagggcccaagcgtcttccccctggcaccctcctccaagagcacctctggcggcacagccgccctgggctgcctggtcaaggactacttccccgaacccgtgaccgtgagctggaactcaggcgccctgaccagcggcgtgcacaccttccccgctgtcctgcagtcctcaggactctactccctcagcagcgtggtgaccgtgccctccagcagcttgggcacccagacctacatctgcaacgtgaatcacaagcccagcaacaccaaggtggacaagaaggttgagcccaaatcttgtgacaaaactcacacatgcccaccctgcccagcacctgaagccgcggggggaccctcagtcttcctcttccccccaaaacccaaggacaccctcatgatctcccggacccctgaggtcacatgcgtggtggtggacgtgagccacgaagaccctgaggtcaagttcaactggtacgtggacggcgtggaggtgcataatgccaagacaaagccccgggaggagcagtacaacagcacgtaccgggtggtcagcgtcctcaccgtcctgcaccaggactggctgaatggcaaggagtacaagtgcaaggtctccaacaaagccctcgcagcccccatcgagaaaaccatctccaaagccaaaggccagccccgggaaccacaggtgtacaccctgcccccatcccgggaggagatgaccaagaaccaggtcagcctgacctgcctggtcaaaggcttctatcccagcgacatcgccgtggagtgggagagcaatggccagcccgagaacaactacaagaccacccctcccgtgctggactccgacggctccttcttcctctacagcaagctcaccgtggacaagagcaggtggcagcagggcaacgtcttctcatgctccgtgatgcatgaggctctgcacaaccactacacccagaagagcctctccctgtctcccggcaaatgagatatcgggcccgtttaaacggg

SEQ ID NO: 20 - protein, 8 aa, synthetic construct
GFTFRDYY

SEQ ID NO: 21 - protein, 8 aa, synthetic construct
IGFDESRT

SEQ ID NO: 22 - protein, 16 aa, synthetic construct
TRHGVSYYSGDNWFAY

SEQ ID NO: 23 - protein, 123 aa, synthetic construct; identical to SEQ ID NO: 15

SEQ ID NO: 24 - protein, 472 aa, synthetic construct
MKHLWFFLLLVAAPRWVLSEVQLVESNGALVQPGRSLKLSCAASGFTFRDYYMAWVRQAPSKGLEWVASIGFDESRTYYRDSVKGRFTISRDDVKSTLYLQLDSLRSEDTATYYCTRHGVSYYSGDNWFAYWGQGALVIVSSASTKGPSVFPLAPSSKSTSGGTAALGCLVKDYFPEPVTVSWNSGALTSGVHTFPAVLQSSGLYSLSSVVTVPSSSLGTQTYICNVNHKPSNTKVDKKVEPKSCDKTHTCPPCPAPEAAGGPSVFLFPPKPKDTLMISRTPEVTCVVVDVSHEDPEVKFNWYVDGVEVHNAKTKPREEQYNSTYRVVSVLTVLHQDWLNGKEYKCKVSNKALAAPIEKTISKAKGQPREPQVYTLPPSREEMTKNQVSLTCLVKGFYPSDIAVEWESNGQPENNYKTTPPVLDSDGSFFLYSKLTVDKSRWQQGNVFSCSVMHEALHNHYTQKSLSLSPGK

SEQ ID NO: 25 - DNA, 1416 bp, synthetic construct
  source 1..1416: mol_type = other DNA
atgaagcacctgtggttctttctgctgctggtggccgcacctagatgggtcctgtctgaagtgcagctggtggaaagcaatggcgccctggttcagcctggcagaagcctgaaactgagctgtgccgccagcggcttcaccttcagagactactatatggcctgggtccgacaggcccctagcaaaggacttgagtgggttgccagcatcggcttcgacgagagccggacctactaccgggatagcgtgaagggcagattcaccatcagccgggacgacgtgaagtctaccctgtacctgcagctggacagcctgagaagcgaggataccgccacctactactgcaccagacacggcgtgtcctactacagcggcgacaattggttcgcctattggggacagggcgctctggtcatcgttagctcagcctccaccaagggcccaagcgtcttccccctggcaccctcctccaagagcacctctggcggcacagccgccctgggctgcctggtcaaggactacttccccgaacccgtgaccgtgagctggaactcaggcgccctgaccagcggcgtgcacaccttccccgctgtcctgcagtcctcaggactctactccctcagcagcgtggtgaccgtgccctccagcagcttgggcacccagacctacatctgcaacgtgaatcacaagcccagcaacaccaaggtggacaagaaggttgagcccaaatcttgtgacaaaactcacacatgcccaccctgcccagcacctgaagccgcggggggaccctcagtcttcctcttccccccaaaacccaaggacaccctcatgatctcccggacccctgaggtcacatgcgtggtggtggacgtgagccacgaagaccctgaggtcaagttcaactggtacgtggacggcgtggaggtgcataatgccaagacaaagccccgggaggagcagtacaacagcacgtaccgggtggtcagcgtcctcaccgtcctgcaccaggactggctgaatggcaaggagtacaagtgcaaggtctccaacaaagccctcgcagcccccatcgagaaaaccatctccaaagccaaaggccagccccgggaaccacaggtgtacaccctgcccccatcccgggaggagatgaccaagaaccaggtcagcctgacctgcctggtcaaaggcttctatcccagcgacatcgccgtggagtgggagagcaatggccagcccgagaacaactacaagaccacccctcccgtgctggactccgacggctccttcttcctctacagcaagctcaccgtggacaagagcaggtggcagcagggcaacgtcttctcatgctccgtgatgcatgaggctctgcacaaccactacacccagaagagcctctccctgtctcccggcaaa

SEQ ID NO: 26 - protein, 12 aa, synthetic construct
QGLLYSGDQKNY

SEQ ID NO: 27 - skipped

SEQ ID NO: 28 - protein, 9 aa, synthetic construct
QQYYDPPYT

SEQ ID NO: 29 - protein, 114 aa, synthetic construct; identical to SEQ ID NO: 17

SEQ ID NO: 30 - protein, 240 aa, synthetic construct
MVLQTQVFISLLLWISGAYGDIVMTQSPSSLAVSAGETVIINCKSSQGLLYSGDQKNYLAWYQQKPGQSPKLLIYWASTRQSGVPDRFIGSGSGTDFTLTISSVQGEDLAIYYCQQYYDPPYTFGAGTKLELKRTVAAPSVFIFPPSDEQLKSGTASVVCLLNNFYPREAKVQWKVDNALQSGNSQESVTEQDSKDSTYSLSSTLTLSKADYEKHKVYACEVTHQGLSSPVTKSFNRGEC

SEQ ID NO: 31 - DNA, 720 bp, synthetic construct
  source 1..720: mol_type = other DNA
atggttctgcagacccaggtgttcatcagcctgctgctgtggatcagcggcgcctatggcgacatcgtgatgacacagagccctagcagcctggctgtgtctgctggcgagacagtgatcatcaactgcaagagcagccagggcctgctgtactccggcgaccagaagaattacctggcctggtatcagcagaagcccggacagtctcccaagctgctgatctactgggccagcacaagacagagcggcgtgcccgatagattcatcggctctggcagcggcaccgacttcaccctgacaatcagtagcgtgcagggcgaagatctggccatctactactgccagcagtactacgaccctccttacacctttggagccggcaccaagctggaactgaagcgtacggtggccgccccctccgtgttcatcttccccccctccgacgagcagctgaagtccggcaccgcctccgtggtgtgcctgctgaataacttctaccccagagaggccaaggtgcagtggaaggtggacaacgccctgcagtccgggaactcccaggagagcgtgaccgagcaggacagcaaggacagcacctacagcctgagcagcaccctgaccctgagcaaagccgactacgagaagcacaaggtgtacgcctgcgaggtgacccaccagggcctgagctcccccgtcaccaagagcttcaacaggggggagtgt

SEQ ID NO: 32 - protein, 8 aa, synthetic construct
GFTFRDYY

SEQ ID NO: 33 - protein, 8 aa, synthetic construct
IGFDESRT

SEQ ID NO: 34 - protein, 16 aa, synthetic construct
TRHGVSYYSGDNWFAY

SEQ ID NO: 35 - protein, 123 aa, synthetic construct
EVQLVESGGGLVQPGGSLRLSCAASGFTFRDYYMAWVRQAPGKGLEWVASIGFDESRTYYADSVKGRFTISRDDSKSTLYLQMNSLRAEDTAVYYCTRHGVSYYSGDNWFAYWGQGTLVTVSS

SEQ ID NO: 36 - protein, 472 aa, synthetic construct
MKHLWFFLLLVAAPRWVLSEVQLVESGGGLVQPGGSLRLSCAASGFTFRDYYMAWVRQAPGKGLEWVASIGFDESRTYYADSVKGRFTISRDDSKSTLYLQMNSLRAEDTAVYYCTRHGVSYYSGDNWFAYWGQGTLVTVSSASTKGPSVFPLAPSSKSTSGGTAALGCLVKDYFPEPVTVSWNSGALTSGVHTFPAVLQSSGLYSLSSVVTVPSSSLGTQTYICNVNHKPSNTKVDKKVEPKSCDKTHTCPPCPAPEAAGGPSVFLFPPKPKDTLMISRTPEVTCVVVDVSHEDPEVKFNWYVDGVEVHNAKTKPREEQYNSTYRVVSVLTVLHQDWLNGKEYKCKVSNKALAAPIEKTISKAKGQPREPQVYTLPPSREEMTKNQVSLTCLVKGFYPSDIAVEWESNGQPENNYKTTPPVLDSDGSFFLYSKLTVDKSRWQQGNVFSCSVMHEALHNHYTQKSLSLSPGK

SEQ ID NO: 37 - DNA, 1416 bp, synthetic construct
  source 1..1416: mol_type = other DNA
atgaagcacctgtggttctttctgctgctggtggccgctcctagatgggtgctgtctgaagtgcagctggtggaatctggcggaggactggttcaacctggcggctctctgagactgtcttgtgccgccagcggcttcaccttccgggattactatatggcctgggtccgacaggcccctggcaaaggacttgaatgggttgccagcatcggcttcgacgagagcagaacctactacgccgacagcgtgaagggcagattcaccatcagccgggacgacagcaagagcaccctgtacctgcagatgaacagcctgagagccgaggacaccgccgtgtactactgtacaagacatggcgtgtcctactacagcggcgacaattggttcgcctattggggccagggcaccctggttacagtgtctagcgcctctacaaagggccccagcgttttcccactggctcctagcagcaagtctaccagcggaggaacagccgctctgggctgtctggtcaaggactactttcccgagcctgtgaccgtgtcctggaattctggcgctctgacaagcggcgtgcacacctttccagctgtgctgcaaagcagcggcctgtactctctgagcagcgtggtcacagtgccaagctctagcctgggcacccagacctacatctgcaatgtgaaccacaagcctagcaacaccaaggtggacaagaaggtggaacccaagagctgcgacaagacccacacctgtcctccatgtcctgctccagaagctgcaggcggcccttccgtgtttctgttccctccaaagcctaaggacaccctgatgatcagcagaacccctgaagtgacctgcgtggtggtggatgtgtcccacgaggatcccgaagtgaagttcaattggtacgtggacggcgtggaagtgcacaacgccaagaccaagcctagagaggaacagtacaacagcacctacagagtggtgtccgtgctgaccgtgctgcaccaggattggctgaacggcaaagagtacaagtgcaaggtgtccaacaaggccctggctgcccctatcgagaaaaccatcagcaaggccaagggccagcctagggaaccccaggtttacacactgcctccaagccgggaagagatgaccaagaaccaggtgtccctgacctgcctggttaagggcttctacccctccgatatcgccgtggaatgggagagcaatggccagccagagaacaactacaagacaacccctcctgtgctggacagcgacggctcattcttcctgtacagcaagctgacagtggacaagtccagatggcagcagggcaacgtgttcagctgcagcgtgatgcacgaggccctgcacaaccactacacccagaagtccctgagcctgtctcctggcaaa

SEQ ID NO: 38 - protein, 8 aa, synthetic construct
GFTFRDYY

SEQ ID NO: 39 - protein, 8 aa, synthetic construct
IGFDESRT

SEQ ID NO: 40 - protein, 16 aa, synthetic construct
ARHGVSYYSGDNWFAY

SEQ ID NO: 41 - protein, 123 aa, synthetic construct
EVQLVESGGGLVQPGGSLRLSCAASGFTFRDYYMAWVRQAPGKGLEWVSSIGFDESRTYYADSVKGRFTISRDDSKNTLYLQMNSLRAEDTAVYYCARHGVSYYSGDNWFAYWGQGTLVTVSS

SEQ ID NO: 42 - protein, 472 aa, synthetic construct
MKHLWFFLLLVAAPRWVLSEVQLVESGGGLVQPGGSLRLSCAASGFTFRDYYMAWVRQAPGKGLEWVSSIGFDESRTYYADSVKGRFTISRDDSKNTLYLQMNSLRAEDTAVYYCARHGVSYYSGDNWFAYWGQGTLVTVSSASTKGPSVFPLAPSSKSTSGGTAALGCLVKDYFPEPVTVSWNSGALTSGVHTFPAVLQSSGLYSLSSVVTVPSSSLGTQTYICNVNHKPSNTKVDKKVEPKSCDKTHTCPPCPAPEAAGGPSVFLFPPKPKDTLMISRTPEVTCVVVDVSHEDPEVKFNWYVDGVEVHNAKTKPREEQYNSTYRVVSVLTVLHQDWLNGKEYKCKVSNKALAAPIEKTISKAKGQPREPQVYTLPPSREEMTKNQVSLTCLVKGFYPSDIAVEWESNGQPENNYKTTPPVLDSDGSFFLYSKLTVDKSRWQQGNVFSCSVMHEALHNHYTQKSLSLSPGK

SEQ ID NO: 43 - DNA, 1416 bp, synthetic construct
  source 1..1416: mol_type = other DNA
atgaaacacctgtggttcttcctcctgctggtggcagctcccagatgggtgctgagcgaggtgcagctggttgaatctggcggaggactggttcagcctggcggatctctgagactgtcttgtgccgccagcggcttcaccttccgggattactatatggcctgggtccgacaggcccctggcaaaggacttgaatgggtgtccagcatcggcttcgacgagagcagaacctactacgccgacagcgtgaagggcagattcaccatcagccgggacgacagcaagaacaccctgtacctgcagatgaacagcctgagagccgaggacaccgccgtgtactattgtgccagacatggcgtgtcctactacagcggcgacaattggttcgcctattggggccagggcaccctggttacagtgagctcagcctccaccaagggcccaagcgtcttccccctggcaccctcctccaagagcacctctggcggcacagccgccctgggctgcctggtcaaggactacttccccgaacccgtgaccgtgagctggaactcaggcgccctgaccagcggcgtgcacaccttccccgctgtcctgcagtcctcaggactctactccctcagcagcgtggtgaccgtgccctccagcagcttgggcacccagacctacatctgcaacgtgaatcacaagcccagcaacaccaaggtggacaagaaggttgagcccaaatcttgtgacaaaactcacacatgcccaccctgcccagcacctgaagccgcggggggaccctcagtcttcctcttccccccaaaacccaaggacaccctcatgatctcccggacccctgaggtcacatgcgtggtggtggacgtgagccacgaagaccctgaggtcaagttcaactggtacgtggacggcgtggaggtgcataatgccaagacaaagccccgggaggagcagtacaacagcacgtaccgggtggtcagcgtcctcaccgtcctgcaccaggactggctgaatggcaaggagtacaagtgcaaggtctccaacaaagccctcgcagcccccatcgagaaaaccatctccaaagccaaaggccagccccgggaaccacaggtgtacaccctgcccccatcccgggaggagatgaccaagaaccaggtcagcctgacctgcctggtcaaaggcttctatcccagcgacatcgccgtggagtgggagagcaatggccagcccgagaacaactacaagaccacccctcccgtgctggactccgacggctccttcttcctctacagcaagctcaccgtggacaagagcaggtggcagcagggcaacgtcttctcatgctccgtgatgcatgaggctctgcacaaccactacacccagaagagcctctccctgtctcccggcaaa

SEQ ID NO: 44 - protein, 8 aa, synthetic construct
GFTFRDYY

SEQ ID NO: 45 - protein, 8 aa, synthetic construct
IGFDESRT

SEQ ID NO: 46 - protein, 16 aa, synthetic construct
ARHGVSKYSGDNWFAY

SEQ ID NO: 47 - protein, 123 aa, synthetic construct
EVQLVESGGGLVQPGGSLRLSCAASGFTFRDYYMAWVRQAPGKGLEWVSSIGFDESRTYYADSVKGRFTISRDDSKNTLYLQMNSLRAEDTAVYYCARHGVSKYSGDNWFAYWGQGTLVTVSS

SEQ ID NO: 48 - protein, 472 aa, synthetic construct
MKHLWFFLLLVAAPRWVLSEVQLVESGGGLVQPGGSLRLSCAASGFTFRDYYMAWVRQAPGKGLEWVSSIGFDESRTYYADSVKGRFTISRDDSKNTLYLQMNSLRAEDTAVYYCARHGVSKYSGDNWFAYWGQGTLVTVSSASTKGPSVFPLAPSSKSTSGGTAALGCLVKDYFPEPVTVSWNSGALTSGVHTFPAVLQSSGLYSLSSVVTVPSSSLGTQTYICNVNHKPSNTKVDKKVEPKSCDKTHTCPPCPAPEAAGGPSVFLFPPKPKDTLMISRTPEVTCVVVDVSHEDPEVKFNWYVDGVEVHNAKTKPREEQYNSTYRVVSVLTVLHQDWLNGKEYKCKVSNKALAAPIEKTISKAKGQPREPQVYTLPPSREEMTKNQVSLTCLVKGFYPSDIAVEWESNGQPENNYKTTPPVLDSDGSFFLYSKLTVDKSRWQQGNVFSCSVMHEALHNHYTQKSLSLSPGK

SEQ ID NO: 49 - DNA, 1416 bp, synthetic construct
  source 1..1416: mol_type = other DNA
atgaaacacctgtggttcttcctcctgctggtggcagctcccagatgggtgctgagcgaggtgcagctggttgaatctggcggaggactggttcagcctggcggatctctgagactgtcttgtgccgccagcggcttcaccttccgggattactatatggcctgggtccgacaggcccctggcaaaggacttgaatgggtgtccagcatcggcttcgacgagagcagaacctactacgccgacagcgtgaagggcagattcaccatcagccgggacgacagcaagaacaccctgtacctgcagatgaacagcctgagagccgaggacaccgccgtgtactattgtgccagacatggcgtgtccaaatacagcggcgacaattggttcgcctattggggccagggcaccctggttacagtgagctcagcctccaccaagggcccaagcgtcttccccctggcaccctcctccaagagcacctctggcggcacagccgccctgggctgcctggtcaaggactacttccccgaacccgtgaccgtgagctggaactcaggcgccctgaccagcggcgtgcacaccttccccgctgtcctgcagtcctcaggactctactccctcagcagcgtggtgaccgtgccctccagcagcttgggcacccagacctacatctgcaacgtgaatcacaagcccagcaacaccaaggtggacaagaaggttgagcccaaatcttgtgacaaaactcacacatgcccaccctgcccagcacctgaagccgcggggggaccctcagtcttcctcttccccccaaaacccaaggacaccctcatgatctcccggacccctgaggtcacatgcgtggtggtggacgtgagccacgaagaccctgaggtcaagttcaactggtacgtggacggcgtggaggtgcataatgccaagacaaagccccgggaggagcagtacaacagcacgtaccgggtggtcagcgtcctcaccgtcctgcaccaggactggctgaatggcaaggagtacaagtgcaaggtctccaacaaagccctcgcagcccccatcgagaaaaccatctccaaagccaaaggccagccccgggaaccacaggtgtacaccctgcccccatcccgggaggagatgaccaagaaccaggtcagcctgacctgcctggtcaaaggcttctatcccagcgacatcgccgtggagtgggagagcaatggccagcccgagaacaactacaagaccacccctcccgtgctggactccgacggctccttcttcctctacagcaagctcaccgtggacaagagcaggtggcagcagggcaacgtcttctcatgctccgtgatgcatgaggctctgcacaaccactacacccagaagagcctctccctgtctcccggcaaa

SEQ ID NO: 50 - protein, 8 aa, synthetic construct
GFTFRDYY

SEQ ID NO: 51 - protein, 8 aa, synthetic construct
IGFDESRT

SEQ ID NO: 52 - protein, 16 aa, synthetic construct
ARHGVSRYSGDNWFAY

SEQ ID NO: 53 - protein, 123 aa, synthetic construct
EVQLVESGGGLVQPGGSLRLSCAASGFTFRDYYMAWVRQAPGKGLEWVSSIGFDESRTYYADSVKGRFTISRDDSKNTLYLQMNSLRAEDTAVYYCARHGVSRYSGDNWFAYWGQGTLVTVSS

SEQ ID NO: 54 - protein, 472 aa, synthetic construct
MKHLWFFLLLVAAPRWVLSEVQLVESGGGLVQPGGSLRLSCAASGFTFRDYYMAWVRQAPGKGLEWVSSIGFDESRTYYADSVKGRFTISRDDSKNTLYLQMNSLRAEDTAVYYCARHGVSRYSGDNWFAYWGQGTLVTVSSASTKGPSVFPLAPSSKSTSGGTAALGCLVKDYFPEPVTVSWNSGALTSGVHTFPAVLQSSGLYSLSSVVTVPSSSLGTQTYICNVNHKPSNTKVDKKVEPKSCDKTHTCPPCPAPEAAGGPSVFLFPPKPKDTLMISRTPEVTCVVVDVSHEDPEVKFNWYVDGVEVHNAKTKPREEQYNSTYRVVSVLTVLHQDWLNGKEYKCKVSNKALAAPIEKTISKAKGQPREPQVYTLPPSREEMTKNQVSLTCLVKGFYPSDIAVEWESNGQPENNYKTTPPVLDSDGSFFLYSKLTVDKSRWQQGNVFSCSVMHEALHNHYTQKSLSLSPGK

SEQ ID NO: 55 - DNA, 1416 bp, synthetic construct
  source 1..1416: mol_type = other DNA
atgaaacacctgtggttcttcctcctgctggtggcagctcccagatgggtgctgagcgaggtgcagctggttgaatctggcggaggactggttcagcctggcggatctctgagactgtcttgtgccgccagcggcttcaccttccgggattactatatggcctgggtccgacaggcccctggcaaaggacttgaatgggtgtccagcatcggcttcgacgagagcagaacctactacgccgacagcgtgaagggcagattcaccatcagccgggacgacagcaagaacaccctgtacctgcagatgaacagcctgagagccgaggacaccgccgtgtactattgtgccagacatggcgtgtccagatacagcggcgacaattggttcgcctattggggccagggcaccctggttacagtgagctcagcctccaccaagggcccaagcgtcttccccctggcaccctcctccaagagcacctctggcggcacagccgccctgggctgcctggtcaaggactacttccccgaacccgtgaccgtgagctggaactcaggcgccctgaccagcggcgtgcacaccttccccgctgtcctgcagtcctcaggactctactccctcagcagcgtggtgaccgtgccctccagcagcttgggcacccagacctacatctgcaacgtgaatcacaagcccagcaacaccaaggtggacaagaaggttgagcccaaatcttgtgacaaaactcacacatgcccaccctgcccagcacctgaagccgcggggggaccctcagtcttcctcttccccccaaaacccaaggacaccctcatgatctcccggacccctgaggtcacatgcgtggtggtggacgtgagccacgaagaccctgaggtcaagttcaactggtacgtggacggcgtggaggtgcataatgccaagacaaagccccgggaggagcagtacaacagcacgtaccgggtggtcagcgtcctcaccgtcctgcaccaggactggctgaatggcaaggagtacaagtgcaaggtctccaacaaagccctcgcagcccccatcgagaaaaccatctccaaagccaaaggccagccccgggaaccacaggtgtacaccctgcccccatcccgggaggagatgaccaagaaccaggtcagcctgacctgcctggtcaaaggcttctatcccagcgacatcgccgtggagtgggagagcaatggccagcccgagaacaactacaagaccacccctcccgtgctggactccgacggctccttcttcctctacagcaagctcaccgtggacaagagcaggtggcagcagggcaacgtcttctcatgctccgtgatgcatgaggctctgcacaaccactacacccagaagagcctctccctgtctcccggcaaa

SEQ ID NO: 56 - protein, 12 aa, synthetic construct
QGLLYSGDQKNY

SEQ ID NO: 57 - skipped

SEQ ID NO: 58 - protein, 9 aa, synthetic construct
QQYYDPPYT

SEQ ID NO: 59 - protein, 114 aa, synthetic construct
DIQMTQSPSSLSASVGDRVTITCKSSQGLLYSGDQKNYLAWYQQKPGKSPKLLIYWASTRQSGVPDRFSGSGSGTDFTLTISSLQPEDFATYYCQQYYDPPYTFGQGTKVEIKR

SEQ ID NO: 60 - protein, 240 aa, synthetic construct
MVLQTQVFISLLLWISGAYGDIQMTQSPSSLSASVGDRVTITCKSSQGLLYSGDQKNYLAWYQQKPGKSPKLLIYWASTRQSGVPDRFSGSGSGTDFTLTISSLQPEDFATYYCQQYYDPPYTFGQGTKVEIKRTVAAPSVFIFPPSDEQLKSGTASVVCLLNNFYPREAKVQWKVDNALQSGNSQESVTEQDSKDSTYSLSSTLTLSKADYEKHKVYACEVTHQGLSSPVTKSFNRGEC

SEQ ID NO: 61 - DNA, 720 bp, synthetic construct
  source 1..720: mol_type = other DNA
atggtgctgcagacccaggtgttcatctccctgctgctgtggatctccggcgcgtacggcgacatccagatgacacagagccctagcagcctgtctgccagcgtgggagacagagtgaccatcacatgcaagagcagccagggcctgctgtactccggcgaccagaagaattacctggcctggtatcagcagaagcccggcaagtctcccaagctgctgatctactgggccagcacaagacagagcggcgtgcccgatagattttctggcagcggctctggcaccgacttcaccctgaccatatctagcctgcagcctgaggacttcgccacctactactgccagcagtactacgaccctccttacacctttggccagggcaccaaggtggaaatcaagcgtacggtggccgccccctccgtgttcatcttccccccctccgacgagcagctgaagtccggcaccgcctccgtggtgtgcctgctgaataacttctaccccagagaggccaaggtgcagtggaaggtggacaacgccctgcagtccgggaactcccaggagagcgtgaccgagcaggacagcaaggacagcacctacagcctgagcagcaccctgaccctgagcaaagccgactacgagaagcacaaggtgtacgcctgcgaggtgacccaccagggcctgagctcccccgtcaccaagagcttcaacaggggggagtgt

SEQ ID NO: 62 - protein, 12 aa, synthetic construct
QGLLYSGDQKNY

SEQ ID NO: 63 - skipped

SEQ ID NO: 64 - protein, 9 aa, synthetic construct
QQYYDPPYT

SEQ ID NO: 65 - protein, 114 aa, synthetic construct
DIQMTQSPSSLSASVGDRVTITCKSSQGLLYSGDQKNYLAWYQQKPGKAPKLLIYWASTRQSGVPSRFSGSGSGTDFTLTISSLQPEDFATYYCQQYYDPPYTFGQGTKVEIKR

SEQ ID NO: 66 - protein, 240 aa, synthetic construct
MVLQTQVFISLLLWISGAYGDIQMTQSPSSLSASVGDRVTITCKSSQGLLYSGDQKNYLAWYQQKPGKAPKLLIYWASTRQSGVPSRFSGSGSGTDFTLTISSLQPEDFATYYCQQYYDPPYTFGQGTKVEIKRTVAAPSVFIFPPSDEQLKSGTASVVCLLNNFYPREAKVQWKVDNALQSGNSQESVTEQDSKDSTYSLSSTLTLSKADYEKHKVYACEVTHQGLSSPVTKSFNRGEC

SEQ ID NO: 67 - DNA, 720 bp, synthetic construct
  source 1..720: mol_type = other DNA
atggtgctgcagacccaggtgttcatctccctgctgctgtggatctccggcgcgtacggcgacatccagatgacacagagccctagcagcctgtctgccagcgtgggagacagagtgaccatcacatgcaagagcagccagggcctgctgtactccggcgaccagaagaattacctggcctggtatcagcagaagcccggcaaggctcctaagctgctgatctactgggccagcacaagacagagcggcgtgccaagcagattttctggcagcggctctggcaccgacttcaccctgaccatatctagcctgcagcctgaggacttcgccacctactactgccagcagtactacgaccctccttacacctttggccagggcaccaaggtggaaatcaagcgtacggtggccgccccctccgtgttcatcttccccccctccgacgagcagctgaagtccggcaccgcctccgtggtgtgcctgctgaataacttctaccccagagaggccaaggtgcagtggaaggtggacaacgccctgcagtccgggaactcccaggagagcgtgaccgagcaggacagcaaggacagcacctacagcctgagcagcaccctgaccctgagcaaagccgactacgagaagcacaaggtgtacgcctgcgaggtgacccaccagggcctgagctcccccgtcaccaagagcttcaacaggggggagtgt

SEQ ID NO: 68 - protein, 469 aa, synthetic construct
MKHLWFFLLLVAAPRWVLSEVQLVQSGAEVKKPGASVKVSCKASGYKFSSYWIEWVKQAPGQGLEWIGEILPGSDTTNYNEKFKDRATFTSDTSINTAYMELSRLRSDDTAVYYCARDRGNYRAWFGYWGQGTLVTVSSASTKGPSVFPLAPSSKSTSGGTAALGCLVKDYFPEPVTVSWNSGALTSGVHTFPAVLQSSGLYSLSSVVTVPSSSLGTQTYICNVNHKPSNTKVDKKVEPKSCDKTHTCPPCPAPELLGGPSVFLFPPKPKDTLMISRTPEVTCVVVDVSHEDPEVKFNWYVDGVEVHNAKTKPREEQYNSTYRVVSVLTVLHQDWLNGKEYKCKVSNKALPAPIEKTISKAKGQPREPQVYTLPPSREEMTKNQVSLTCLVKGFYPSDIAVEWESNGQPENNYKTTPPVLDSDGSFFLYSKLTVDKSRWQQGNVFSCSVMHEALHNHYTQKSLSLSPGK

SEQ ID NO: 69 - DNA, 1407 bp, synthetic construct
  source 1..1407: mol_type = other DNA
atgaaacacctgtggttcttcctcctgctggtggcagctcccagatgggtgctgagcgaagttcagctggttcagtctggcgccgaagtgaagaaacctggcgcctctgtgaaggtgtcctgcaaggccagcggctacaagttcagcagctactggatcgagtgggtcaagcaggcccctggacaaggcctggaatggatcggagagatcctgcctggcagcgacaccaccaactacaacgagaagttcaaggaccgggccaccttcacctccgacacctctatcaacaccgcctacatggaactgagccggctgagatccgatgacaccgccgtgtactactgcgccagagacagaggcaactacagagcttggtttggctactggggccagggcacactggtcacagttagctcagcctccaccaagggcccaagcgtcttccccctggcaccctcctccaagagcacctctggcggcacagccgccctgggctgcctggtcaaggactacttccccgaacccgtgaccgtgagctggaactcaggcgccctgaccagcggcgtgcacaccttccccgctgtcctgcagtcctcaggactctactccctcagcagcgtggtgaccgtgccctccagcagcttgggcacccagacctacatctgcaacgtgaatcacaagcccagcaacaccaaggtggacaagaaggttgagcccaaatcttgtgacaaaactcacacatgcccaccctgcccagcacctgaactcctggggggaccctcagtcttcctcttccccccaaaacccaaggacaccctcatgatctcccggacccctgaggtcacatgcgtggtggtggacgtgagccacgaagaccctgaggtcaagttcaactggtacgtggacggcgtggaggtgcataatgccaagacaaagccccgggaggagcagtacaacagcacgtaccgggtggtcagcgtcctcaccgtcctgcaccaggactggctgaatggcaaggagtacaagtgcaaggtctccaacaaagccctcccagcccccatcgagaaaaccatctccaaagccaaaggccagccccgggaaccacaggtgtacaccctgcccccatcccgggaggagatgaccaagaaccaggtcagcctgacctgcctggtcaaaggcttctatcccagcgacatcgccgtggagtgggagagcaatggccagcccgagaacaactacaagaccacccctcccgtgctggactccgacggctccttcttcctctacagcaagctcaccgtggacaagagcaggtggcagcagggcaacgtcttctcatgctccgtgatgcatgaggctctgcacaaccactacacccagaagagcctctccctgtctcccggcaaa

SEQ ID NO: 70 - protein, 234 aa, synthetic construct
MVLQTQVFISLLLWISGAYGDIQMTQSPSSLSASVGDRVTITCRASQDISNYLNWYQQKPGGAVKFLIYYTSRLHSGVPSRFSGSGSGTDYTLTISSLQPEDFATYFCQQGEALPWTFGGGTKVEIKRTVAAPSVFIFPPSDEQLKSGTASVVCLLNNFYPREAKVQWKVDNALQSGNSQESVTEQDSKDSTYSLSSTLTLSKADYEKHKVYACEVTHQGLSSPVTKSFNRGEC

SEQ ID NO: 71 - DNA, 702 bp, synthetic construct
  source 1..702: mol_type = other DNA
atggtgctgcagacccaggtgttcatctccctgctgctgtggatctccggcgcgtacggcgatatccagatgacacagagccctagcagcctgtctgccagcgtgggagacagagtgaccatcacctgtagagccagccaggacatcagcaactacctgaactggtatcagcagaaacccggcggagccgtgaagttcctgatctactacaccagcagactgcacagcggcgtgcccagcagattttctggctctggcagcggcaccgactacaccctgaccatatctagcctgcagcctgaggacttcgctacctacttctgccagcaaggcgaagccctgccttggacatttggcggcggaacaaaggtggaaatcaagcgtacggtggccgccccctccgtgttcatcttccccccctccgacgagcagctgaagtccggcaccgcctccgtggtgtgcctgctgaataacttctaccccagagaggccaaggtgcagtggaaggtggacaacgccctgcagtccgggaactcccaggagagcgtgaccgagcaggacagcaaggacagcacctacagcctgagcagcaccctgaccctgagcaaagccgactacgagaagcacaaggtgtacgcctgcgaggtgacccaccagggcctgagctcccccgtcaccaagagcttcaacaggggggagtgt

SEQ ID NO: 72 - protein, 474 aa, Homo sapiens
MKHLWFFLLLVAAPRWVLSQVQLVQSGAEVKKPGASVKVSCKASGYTFTSYWINWVRQAPGQGLEWMGNIYPGSSSINYNEKFKSRVTITADTSTSTAYMELSSLRSEDTAVYYCARTIYNYGSSGYNYAMDYWGQGTLVTVSSASTKGPSVFPLAPSSKSTSGGTAALGCLVKDYFPEPVTVSWNSGALTSGVHTFPAVLQSSGLYSLSSVVTVPSSSLGTQTYICNVNHKPSNTKVDKKVEPKSCDKTHTCPPCPAPEAAGGPSVFLFPPKPKDTLMISRTPEVTCVVVDVSHEDPEVKFNWYVDGVEVHNAKTKPREEQYNSTYRVVSVLTVLHQDWLNGKEYKCKVSNKALAAPIEKTISKAKGQPREPQVYTLPPSREEMTKNQVSLTCLVKGFYPSDIAVEWESNGQPENNYKTTPPVLDSDGSFFLYSKLTVDKSRWQQGNVFSCSVMHEALHNHYTQKSLSLSPGK

SEQ ID NO: 73 - protein, 234 aa, synthetic construct
MVLQTQVFISLLLWISGAYGDIVMTQSPDSLAVSLGERATINCKASENVGNSVSWYQQKPGQPPKLLIYGASNRYTGVPDRFSGSGSGTDFTLTISSLQAEDVAVYYCGQSYSYPYTFGQGTKVEIKRTVAAPSVFIFPPSDEQLKSGTASVVCLLNNFYPREAKVQWKVDNALQSGNSQESVTEQDSKDSTYSLSSTLTLSKADYEKHKVYACEVTHQGLSSPVTKSFNRGEC